European Patent Specification EP 3 283 657 B1, published June 21, 2023. Title: QUALITY ASSESSMENT OF CIRCULATING CELL-FREE DNA USING MULTIPLEXED DROPLET DIGITAL PCR. Applicant: THE TRANSLATIONAL GENOMICS RESEARCH INSTITUTE. The sequence listing filed with the application follows.

SEQUENCE LISTING (27 sequences)

SEQ ID NO: 1 - DNA, 22 bp, Artificial Sequence
  Primer
tctatgctccctctgtgttaga

SEQ ID NO: 2 - DNA, 24 bp, Artificial Sequence
  Probe
agcaaggtgccctgagaagacaat

SEQ ID NO: 3 - DNA, 20 bp, Artificial Sequence
  Primer
tccaggaattcacccgaaac

SEQ ID NO: 4 - DNA, 23 bp, Artificial Sequence
  Primer
cagacaagatgaggaggtacaaa

SEQ ID NO: 5 - DNA, 24 bp, Artificial Sequence
  Probe
attgagcctgtgcctggctagaaa

SEQ ID NO: 6 - DNA, 21 bp, Artificial Sequence
  Primer
agctgtgagtagaggagtctt

SEQ ID NO: 7 - DNA, 22 bp, Artificial Sequence
  Primer
aaagaggtcttgccaggtattc

SEQ ID NO: 8 - DNA, 24 bp, Artificial Sequence
  Probe
atagggcttcaggccaaacatggt

SEQ ID NO: 9 - DNA, 20 bp, Artificial Sequence
  Primer
agctcactgcagccttaatc

SEQ ID NO: 10 - DNA, 22 bp, Artificial Sequence
  Primer
gtctccaggatagctgcttatg

SEQ ID NO: 11 - DNA, 24 bp, Artificial Sequence
  Probe
tttgggactggcctttgaagctct

SEQ ID NO: 12 - DNA, 18 bp, Artificial Sequence
  Primer
tgcatgtgagcaccaagt

SEQ ID NO: 13 - DNA, 22 bp, Artificial Sequence
  Primer
cttgtacctggtgttcggttat

SEQ ID NO: 14 - DNA, 25 bp, Artificial Sequence
  Probe
agcctctctcctctgcaacctgata

SEQ ID NO: 15 - DNA, 20 bp, Artificial Sequence
  Primer
gtaggctgggtagccaaatc

SEQ ID NO: 16 - DNA, 20 bp, Artificial Sequence
  Primer
ccagcccaagatggatgaat

SEQ ID NO: 17 - DNA, 23 bp, Artificial Sequence
  Probe
tgcagttgttccgaggtgacaca

SEQ ID NO: 18 - DNA, 23 bp, Artificial Sequence
  Primer
ctcttctttcctttcagcaacac

SEQ ID NO: 19 - DNA, 21 bp, Artificial Sequence
  Primer
gcggtggaagtcattctgata

SEQ ID NO: 20 - DNA, 26 bp, Artificial Sequence
  Probe
tggagttggcattggaagcttattct

SEQ ID NO: 21 - DNA, 22 bp, Artificial Sequence
  Primer
tctctctctctccagtgaacaa

SEQ ID NO: 22 - DNA, 20 bp, Artificial Sequence
  Primer
gagggccacagattggtatt

SEQ ID NO: 23 - DNA, 26 bp, Artificial Sequence
  Probe
aatgagatacgagggttgttgctggg

SEQ ID NO: 24 - DNA, 24 bp, Artificial Sequence
  Primer
gatcacttagctcaggaaacaaac

SEQ ID NO: 25 - DNA, 22 bp, Artificial Sequence
  Primer
actgaaaggtcagattcaggag

SEQ ID NO: 26 - DNA, 23 bp, Artificial Sequence
  Probe
atcgccttgatcaacagcctcca

SEQ ID NO: 27 - DNA, 20 bp, Artificial Sequence
  Primer
taccggtttgtgtccaagag